European Patent Specification EP 2 954 064 B1, published January 15, 2025. Title: Protein. Applicant: Green Biologics Limited. The sequence listing filed with the application follows.

SEQUENCE LISTING (5 sequences)

SEQ ID NO: 1 - protein, 674 aa, Clostridium saccharoperbutylacetonicum
MFRRKFNKVILSILVATIVSSTNMFMSGSKAQAAIGNLSENDTIYQIMVDRFYDGDKTNNATGDAFRNTENLEDDFRYMHGGDWQGVIDKLDYIKGMGYSAIWISPVAEPQMWSRADGTGKVWPTAYHGYNVKDPNKANPYFGTKEKLKELVDKAHEKGIKVIIDIVPNHVGDYMLGKQAYYDIKGFEPAAPFNNPNWYHHNGDIDWSREHSDPQMLDDHDLGGLDDLNQDNSDAKAAMNNAIKSWFDYTGADAARVDAAKCMKPSYINELQKYIGVNTFGENFDMNVDFVKKWVGSDAEWGMLDFPLYQAINNDFASGQSFDDMSSSGTCSIKNILAQDNKYNGYANHMVTFIDNHDRNRFLTVANGNVKKLQNALVFMFTVRGVPTVFQGTEQNKGNANGASINGIADTWNRWSMVKKDYNGNVITDYFNENTDTYKLINKLNSFRQKYEALREGTQREMWSSPHLYAFSRRMDSGENVGQEVVNVFNNSDGDQSATIPIRAESTIKVGDKFVNLFDVNDSITVQQGGVTGKQISVNLGENSGKIYVVNNETPNPDQKNVQYKVSYKNTNAQKVTLHYGTNGWKNIQDVNMTKNSNGEFEATITVNNNDILNYCIHIISPTDYWDNNGGQNWNVKVTKAEDYINDGVKSNLKSVNTTTSAAIDSGIDSTVNR

SEQ ID NO: 2 - DNA, 2025 bp, Clostridium saccharoperbutylacetonicum
atgtttagaagaaaatttaacaaggtaatattatctatcttagttgcaacaattgtttcaagcactaacatgtttatgagtggaagcaaggcacaagcggcaattggaaatctaagtgaaaacgatactatttatcaaattatggtagacagattttatgatggagataaaacaaataatgctacaggagatgcatttcgtaatacagaaaatcttgaagatgattttagatatatgcacggcggagattggcaaggtgttattgataagttagattatattaagggcatgggatactcagccatttggatatcaccggttgcggaaccacaaatgtggtctagagctgatggcacaggaaaagtatggcctacagcttatcatggatataatgtgaaagatcccaataaggcaaatccttattttggaacaaaagaaaagctaaaggagttagtagataaagctcacgaaaaggggattaaagtaataatagatatagttccaaatcatgttggggattatatgttaggaaaacaagcttattatgacatcaaggggtttgagccggcagcaccttttaataatccaaattggtatcatcataatggcgatattgattggtcaagagaacactctgatccccaaatgttagatgatcatgatttgggcggtttagatgatttaaatcaagataattctgatgctaaggcagctatgaataatgctattaagtcatggtttgattatactggagctgatgcagcaagggttgacgcagcaaaatgtatgaaaccatcttatattaacgagttacaaaagtatataggagttaatacttttggagaaaattttgatatgaatgtagattttgtgaagaagtgggttggatccgatgcagaatggggaatgctagattttccattatatcaagcaataaataatgattttgcatcaggacaatcttttgatgacatgtcatcatcaggtacttgctctattaaaaatattttagcacaagacaataaatataatggttatgcaaatcatatggtgacttttatagataatcatgatcgtaatagatttttaacagtagcaaatggtaatgtaaaaaaacttcaaaatgcacttgttttcatgtttactgtaagaggggtaccaacagtatttcaaggtacagaacaaaacaaaggtaatgcaaatggagcaagtataaatggtattgcagatacatggaatcgttggtcaatggttaaaaaggattacaatggaaatgtaattacagattattttaatgagaatacagatacttataaactaattaacaaattgaattcatttaggcaaaaatatgaagccttaagagaaggtactcaaagagaaatgtggtcttcaccacatttatatgcattctcaagaaggatggattcaggagaaaatgttggacaagaagttgtaaatgtatttaataattcagatggagatcaaagtgcgaccattccaattagagctgaaagtactataaaagttggagataaatttgtaaatctttttgatgtaaatgattcgatcacagttcaacaaggaggtgttacaggaaaacaaatatcagtgaatttaggagaaaatagtgggaagatttatgttgttaataatgaaacaccaaatccagatcaaaagaacgtacaatataaagtttcatataagaatactaatgcacaaaaagtaacacttcattatggaactaatggatggaaaaacattcaagatgtaaatatgactaagaattccaatggagaatttgaagcaactattacagtaaataataatgatattctaaattactgtattcatattatttcaccaacagactattgggataataatggtggacagaattggaatgtaaaagtgactaaggcagaagattatataaatgatggtgtaaagagtaatttgaagagcgttaatacaactacatcagcagctatagactctgggattgatagtactgtaaatcgttaa

SEQ ID NO: 3 - protein, 674 aa, Clostridium saccharoperbutylacetonicum
MFRRKFNKVILSILVATIVSSTNMFMSGSKAQAAIGNLSENDTIYQIMVDRFYDGDKTNNATGDAFRNTENLEDDFRYMHGGDWQGVIDKLDYIKGMGYSAIWISPVAEPQMWSRADGTGKVWPTAYHGYNVKDPNKANPYFGTKEKLKELVDKAHEKGIKVIIDIVPNHVGDYMLGKQAYYDIKGFEPAAPFNNPNWYHHNGDIDWSREHSDPQMLDDHDLGGLDDLNQDNSDAKAAMNNAIKSWFDYTGADAARVDAAKCMKPSYINELQKYIGVNTFGENFDMNVDFVKKWVGSDAEWGMLDFPLYQAINNDFASGQSFDDMSSSGTCSIKNILAQDNKYNGYANHMVTFIDNHDRNRFLTVANGNVKKLQNALVFMFTVRGVPTVFQGTEQNKGNGNGAILNGIADTWNRWSMVKKDYNGNIITDYFNENTDTYKLISKLNSFRQKYEALREGTQREMWSSPHLYAFSRRMDSGENVGQEVVNVFNNSDGDQSATIPIRAESTIKVGDKLVNLFDVNDSITVQQGGVTGKQISVNLGENSGKIYVVNNETPNPDQKNVQYKVSYKNTNAQKVTLHYGTNGWKNIQDVNMTKNSNGEFEATITVNNNDILNYCIHIISPTDYWDNNGGQNWNVKVTKAEDYINDGVKSNLKSVNTTTSAAIESGIDSTVNR

SEQ ID NO: 4 - DNA, 2025 bp, Clostridium saccharoperbutylacetonicum
atgtttagaagaaaatttaacaaggtaatattatctattttagttgcaacaattgtttcaagcactaacatgtttatgagtggaagcaaggcacaagcggcaattggaaatttaagtgaaaacgatactatttatcaaattatggtagacagattttatgatggagataaaacaaataatgctacaggagatgcatttcgtaatacagaaaatcttgaagatgattttagatatatgcacggcggagattggcaaggtgttattgataagttagattatattaagggcatgggatactcagccatttggatatcaccggttgcggaaccacaaatgtggtctagagctgatggcacaggaaaagtatggcctacagcttaccatggatataatgtgaaagatcccaataaggcaaatccttattttggaacaaaagaaaagctaaaggagttagtagataaagctcacgaaaaggggattaaagtaataatagatatagttccaaatcatgttggggattatatgttaggaaaacaagcttattatgacatcaaggggtttgagccggcagcaccttttaataatccaaattggtatcatcataatggcgatattgattggtcaagagaacactctgatccccaaatgttagatgatcatgatttgggcggtttagatgatttaaatcaagataattctgatgctaaggcagctatgaataatgctattaagtcatggtttgattatactggagctgatgcagcaagggttgacgcagcaaaatgtatgaaaccatcttatattaacgagttacaaaagtatataggagttaatacttttggagaaaattttgatatgaatgtagattttgtgaagaagtgggttggatccgatgcagaatggggaatgctagattttccattatatcaagcaataaataatgattttgcatcaggacaatcttttgatgacatgtcatcatcaggtacttgctctattaaaaatattttagcacaagacaataaatataatggttatgcaaatcatatggtgacttttatagataatcatgatcgtaatagatttttaacagtagcaaatggtaatgttaaaaaacttcaaaatgcacttgttttcatgtttactgtaagaggggtaccaacagtatttcaaggtacagaacaaaacaaaggtaatggaaatggagcaattctaaatggtattgcagatacatggaatcgttggtcaatggttaaaaaggactataatggaaatataattacagattattttaatgagaatacagatacttataaactaattagcaaattgaattcatttaggcaaaaatatgaagccttaagagaaggtactcaaagagaaatgtggtcttcaccacatttatatgcattctcaagaaggatggattcaggagaaaatgttggacaagaagttgtaaatgtatttaataattcagatggagatcaaagtgcgaccattccaattagagctgaaagtactataaaagttggagataaacttgtaaatctttttgatgtaaatgattcgatcacagttcaacaaggaggtgttacaggaaaacaaatatcagtgaatttaggagaaaatagtgggaagatttatgttgttaataatgaaacaccaaatccagatcaaaagaacgtacaatataaagtttcatataagaatactaatgcacaaaaagtaacacttcattatggaactaatggatggaaaaacattcaagatgtaaatatgactaagaattccaatggagaatttgaagcaactattacagtaaataataatgatattctaaattactgtattcatattatttcaccaacagactattgggataataatggtggacagaattggaatgtaaaagtgactaaggcagaagattatataaatgatggtgtaaagagtaatttgaagagcgttaatacaactacatcagcagcgatagaatctggtattgatagtactgtaaatcgttaa

SEQ ID NO: 5 - DNA, 13357 bp, Clostridium saccharoperbutylacetonicum
gttcatggttttttcaataggctagattcacgtataagtaatttaggtgatattagggttatttcattctgagaatttggattttgaatttttttcattaaaatttcagctgccacttcaccaagtttaaatgtatctacatctagacaagttaaggatggagtggtgtaagcagaaaatggttcattgtcaaaagtcacaattccaatatctgtggggctatttaagcccttttctttaagtgctttaagtacaccaaatgcaacataattatttatgcatagtatggcatctatttcaggaaaatctgataataattgaagtgtaagttcataaccactttccttgtctgagttgccttcttttatgtataaattatttttagtaaaatttaatttagaaagtatgtttttataaccaagaagccgattgaaagatattatttcatttgatttgccaccaataaaggctatatttttataaccttgttctattaaatgacatgtggccagttctcctcctacagtattattaacatcaacccagctggtactattcttaaattcctttggctgaccaataaggacataaggaaagtttaaaccgttgagcttactaataatttccgaattgactattgaggtaggtattatgattccatctacttttttactatatatcaatcgatttagaaattctgctttgcattctagtgaatttatgtttgatagggttaactcatagttattgattccaactatactttcaactccaccaataatattatagaaaaagaaatcaagaaaatattcctttctgctaatatctactagaagacctatattaaaactattctggcgagctagctgccttgccgaattatttggaatatagttaagctctttcataatgtttcttactttgagctttgtactttcagaaatagatttatgattatttataactttggataccgttgatttagatacatttgctgcgtgagctatatcatttatagtaactttcatttttaactccttatgtgtgaaattgattatttaaatattataaaacattatttgatttttttcgatatgtacattgttattaataatattactatttattgtaaagtattttagaaattttttatacttctataagtttagcataataatctaaaaatacatatatagttgcacatttcagtgctaaagattaaatttatttatatcatctaaatcctcttaaactcatttaaagttccttctctaaattgaaaaatgaatttccaattgtactcattgcataatttatagatttgttcacaagcataaagactattacctaaaatgtaggtattaagtgttataaacttatattttaattttttcataagtcttttagcatatgccttaataaaacaatatatctggtggaagttaatacaatatattgaaattgattcaatattgcagtatactaaaatgagtaaaccggtttcttaaattttcaatgtatttaaagaatttgtaagacagaagaatataattttcaactttataatatgcttatttgaatgaattaataaaaagatgatttttagtattttgtttataagcctagtagttacaagaagtaaatattttctgtaaaagattataaattaggagggagaattgaaaaatggtaaaaaaaaataaagtattagcatcaatcgtggcagcaactttagttgcaggaacatttgtaggatgtggaggaacaacagctacaagtaataatgctaaagaaattacagtttggtcacatttgaaagaaaaagagattacagagcttactaaagtagcggaaaaatggggaagtgaaaagggagttaaggttaatgttgtagatgataaaggggagatgcaagcatatatacaagccgctaatagttctaaaggtccagatatactttttggtgtacctaatgataacttaggaacatttcaaaaagctggtttactttcagaagtgccaagtggttttatagatgagagtaaatatacatctaaacaagtaatagattcagtgactatagaaggaaaaaaatatgcagttccattagcagctgaaactagtgctctattttataataaagataaagtttcagaagtaccaaaaactatggaagaagttgttgaattaggcaaaaaagtaggatttgaatacgatgtaactgatttatacagaagttatggatttttagcatcgcaaggtagctatatttttaaaaataataatggaactgttgattcaaacgatattggattaggcaatgaaggtgcgataaaaggatatcaattcattcaagatttaattgttaaagacaaattaatgtctcaagatattactgatgatatagctaaagcagatttccaatcaggtaaatcagcattttatatttcaggaccatgggatatagaagcatttaaagattcaggaattaattttggtatagctccaatgccaacattaggtgggaaaactgtttcaacattgatgggagttcaaactgcatttgtaagttcaaagtcacctaatcaagacttatcatgggagttaatgaagtatcttatggaaaatagtgatgacctaatgattaagcaaggaaatagaattccagtttcaaaagcaggtatagaaagtgatgcgtttaaagcggccggaaacatggatgtatttgctaaacaattagaagttgctacagcaatgcctaatattccagaaattcaaactacttggactccggtaaaaaataatataatatctttaataagcggatcaatggattcgaaagaaactgcaaaacaaatagtagatcaaattaaagaaggtataaagcaacaaaaataaaaaagtaaattaagaaaataacatgtagtgctaaagtgattgaaaacaattaactttagcatctttttaatattaatattttcaaaatacacaagccaaaagaagttctctagctatatagtggagtttagtgtacattctatgtaattatattggtaaatgttttcagaaatgtattgaaatccatttaagatggtagtatactaaatagggaaaccggtttacctaatgtaatacatttaaagaaataaaggaatgcgaagacgacgatatttttgatttttatgtgcttattttgatgaaattatgacaaggtaattttataaaatcatttattagtttttcataattatgtgaatgactaataaaaatatataatagtgggggaaagttatgtttagaagaaaatttaacaaggtaatattatctatcttagttgcaacaattgtttcaagcactaacatgtttatgagtggaagcaaggcacaagcggcaattggaaatctaagtgaaaacgatactatttatcaaattatggtagacagattttatgatggagataaaacaaataatgctacaggagatgcatttcgtaatacagaaaatcttgaagatgattttagatatatgcacggcggagattggcaaggtgttattgataagttagattatattaagggcatgggatactcagccatttggatatcaccggttgcggaaccacaaatgtggtctagagctgatggcacaggaaaagtatggcctacagcttatcatggatataatgtgaaagatcccaataaggcaaatccttattttggaacaaaagaaaagctaaaggagttagtagataaagctcacgaaaaggggattaaagtaataatagatatagttccaaatcatgttggggattatatgttaggaaaacaagcttattatgacatcaaggggtttgagccggcagcaccttttaataatccaaattggtatcatcataatggcgatattgattggtcaagagaacactctgatccccaaatgttagatgatcatgatttgggcggtttagatgatttaaatcaagataattctgatgctaaggcagctatgaataatgctattaagtcatggtttgattatactggagctgatgcagcaagggttgacgcagcaaaatgtatgaaaccatcttatattaacgagttacaaaagtatataggagttaatacttttggagaaaattttgatatgaatgtagattttgtgaagaagtgggttggatccgatgcagaatggggaatgctagattttccattatatcaagcaataaataatgattttgcatcaggacaatcttttgatgacatgtcatcatcaggtacttgctctattaaaaatattttagcacaagacaataaatataatggttatgcaaatcatatggtgacttttatagataatcatgatcgtaatagatttttaacagtagcaaatggtaatgtaaaaaaacttcaaaatgcacttgttttcatgtttactgtaagaggggtaccaacagtatttcaaggtacagaacaaaacaaaggtaatgcaaatggagcaagtataaatggtattgcagatacatggaatcgttggtcaatggttaaaaaggattacaatggaaatgtaattacagattattttaatgagaatacagatacttataaactaattaacaaattgaattcatttaggcaaaaatatgaagccttaagagaaggtactcaaagagaaatgtggtcttcaccacatttatatgcattctcaagaaggatggattcaggagaaaatgttggacaagaagttgtaaatgtatttaataattcagatggagatcaaagtgcgaccattccaattagagctgaaagtactataaaagttggagataaatttgtaaatctttttgatgtaaatgattcgatcacagttcaacaaggaggtgttacaggaaaacaaatatcagtgaatttaggagaaaatagtgggaagatttatgttgttaataatgaaacaccaaatccagatcaaaagaacgtacaatataaagtttcatataagaatactaatgcacaaaaagtaacacttcattatggaactaatggatggaaaaacattcaagatgtaaatatgactaagaattccaatggagaatttgaagcaactattacagtaaataataatgatattctaaattactgtattcatattatttcaccaacagactattgggataataatggtggacagaattggaatgtaaaagtgactaaggcagaagattatataaatgatggtgtaaagagtaatttgaagagcgttaatacaactacatcagcagctatagactctgggattgatagtactgtaaatcgttaaatataaatgttaatttaaagaaaaatttcatcatgcatattatatttggcacacaaaaatattaaatatctacttttcgcttctaaatggaaaaaccgcatggttagatcctaaagccttataaaatccatgtttccataattgaagcgaaatataggtagataataatgtataaattaggaggaataattgatgaaaggtgaaataatatatcaaatttttccagacagatttaataaatcaagacaaaataataatgttgaaggtttaaaagaatgggaaagtgaagttgatggacaatgtgttatgggaggtgatttaattggaattaaagagaaacttgattatctatcaaaactcggtgttagtgcaatttatttaaatccaatttttcaggcaaattctaatcataagtatgatactgttaactattataatatagatagttcttttggaactttagatgattttagagaattagtagattcatgtcataaaaaaaatataaaagttattattgatggagtttttaaccatactagcccagatttttttgctttcaaagatatattagaaaatcaagaaagatcaaaatataaggattggtatactatttttagttatccagttaaagtggaaagtccacctaattatagaaattttggaggatgtatagatatgccgcgtcttaatactgaaaatgttgaagttcaaaagtatatagttgatgttattaagtattgggaagggatgaaaatagatggattaagactagatgtaccatattatattgaagactctatgttagaaaaaataagaaaatctactagcttatatatagtaggtgaaatatgggggtgtggcaagaaatttgtgcctcaatattttgatggagtaatgaattattcatttagagatttagtgcaaaaagcagttataagacaaagcattgatgcatcaatattcatagatgaatggaatttcatagaagaaacatacgggcagaatatacattgctgctttaatatgtctggaagtcatgatacagaaaggatttttaatttctgcagaggagatataaagagagaaaaattattctatgcatttttatttttattcccaggaatgcctcttgtatattatggagatgaaataggtatgaaaggagaaaatgacccttattgtagaggaactatggaatggaatgaaagtaaatggaattatgatatatataatcatgtaaaaggtttaatagaacttagaaatagtagtgaagcattgcaaaaagggactatacaatttgttggacataaagaaatgatgtttgcatttgaaagagtgtatgcagaaaaaagagttaaagtatttatgaattttggacatagcaaacagtctattgatggatttgaactagatggtcttagttataaagttatagtttagcattcaaggataactttgcaagttataaaatagcaactttaaacaatcaatgttctttaattggacattggttatcacaatatgtttatctgtttggataaatatatgaataaatttcattaattttatttttttccatgataaaaatcatagagaaaaaggcatatatttaaatttggctttattagtaaattcaattagtataatatattttagtgatattgacataagagattaaataaattatttatataaaaaaagtaagattaagaaatactagatttaaatttttttatatcaaagaggtgggcaattatgaaacaagccaaaacaaaaaaaataacacatactttgaaatcagtgccgtatttattaccagccattatttcaataattatattttcaatattaccaatacttaatacaatatatttggcatttacagactatactatgtattcacaaggaaaaattaattttgtaggaattgcaaattttaaagaagtatttgctggtccatttaaagaagtattttttccggtatttatatggacatgtgtctttgctacattggcaactgcaggaacatttttgttaggactaattatggcaattcttgtaaataatgaaaatataaaagaacgagggctttataaagcaattttaattattccatgggcattaccagctactgttgcaatactttcatggcaaggtttattaaatggaagttatggggcaattaataatttacttataagtgtacatgctatttcagcgcctattccatggttaactaatccattatgggcaagaattgcaataatcatagtaactatatggctaggatttccatatgccatgaatatttgtttgggttcacttcaatcgatacctaaaacatattatgaagcagctgacgttgatggagccagcaagtttgtaaaatttattaaaataactttaccttcgcttgcacaaacagcatatccattagttatttcatcctttgcatttaactttaataattttggtcaagcatatttaattactaatggtaatccggcaagacctggaacacaatttgcaggtttcacagatatattggcttcagtaaattataaattgtcaataacatttggaagatatgaaattgcttccactataagcattattatatttataattttagctacaatttcatacatacaaatgaaagcatcaggacaatttgaggaggttgattaaaatgacatcaaatgcagggaatttgaaattaaataatacagaaggacaaagtgaagaaatacaaaacataaaattaaaatatgtaaaaaaattaagaccagcagaaataagaactgcatggatttcaaggatagtactttggattatgattgtaatagttcttattccaatcatggcagttgtttcagcatctatggctaaaggtaattcatttacgcaaacctctatttttcctaaatcatttactttagagaattatgtaaaagtaataactcaaactaagtttttaatatgggcaagaaattcattagttgtttgttttagcgttgctatgatgcagctaatcatgacaattccagcagcttttgcgttttctaagcttaggtttaaaggtagaaaatttggacttatgacacttttgatattacagatgtttccaaatacaatggcattaccagcaattttaagtgttgcatataatattcggggtggaatggataatttattaccattaatattaattatatcagtaggtagtgcatataacatctggcttatgaagggatacatggatggaattccaaaagaattaactgaaactgcatatatagatggagcaacaacttttcaagctttcattaaggtagtattgccactaataaagaatatgataatagtaatatttatatttgcttttgttggagcttatagcgaatttttatttacatcagctcttataaaagatcaatatacagaaactctagcaacaggtatgcaaggattcattaaagatcatttttcagctaactggactcaatattcagcggctgcaataatggcatcattaccagttgttttgatatcagtattttcacaaaaattctttgcaaaaggattaactgctggatcagtaaaaggctaaagtggggacgtgagtatataatgaagccaactaaggattagaaaataagtagcaattttaataaaattaaaaagtttttctataaaaatctttcaactaaagaaaattcaaaaaacaatgatgtaactattaaaaaatctaaaagtttgcattttaaattattggaaagtatgttctgtatttcaattattccaataataattatttgcagcgttacttttattaaaattaattttattaagtaatgttaattcataagctgaagatgtgaattcagaatcattgattttaaatgataaaagtaaggaattatcgttagctatatctaatgtaaatgagactttaggcaagattgatcttggaactatagattctacaaataatttggaatctttagtgttaaatatggaggaggtatcaaatccaatgatcaaagtagcgtaatagttatatataagtgaaaaggggaaggaattcttatgagattcgaagctgtatatcatagagcctcagataacttatgttattcaattgataaagacaatttaattgtaaatataaagactggttatgatgtagaaaaagtgtttatatattatggtgatccatttgatggaggaattttaggtggcgaatggaaatggaaaggaaaaagagaagaaattccatttaaaaagagattaaagcaccaaatatggtggacaactactttgaaactgaagtataaaagatgtaaatactattttgaattaacggggaatgaagaaacctggttttattttgaagattgttttttaagtgaaaaacaaatgcaattggacggaaaaatgttgcaatgttttacatttccatggatgaatgaagctgatataaataaaacaccagcatgggtaaatgatatggtttggtatcagatattcccagagcgtttttgtaatggaaatccttcaattaatcccaaaggggtccagccttggcataaaggaggcgttacaaatgaagagttttatggtggggatttgcaggggataataaataaattaaattatttaaaagaaataggaattacaggcatatatttaaatccaatattcgaatctccgtcagcacataaatatgatacaactgattatatgaaaatagatcctaattttggagatgaaaatgtatttagaaagcttgtaaataaagcacatgaaaaagggattaggattatgcttgatggagtgtttaatcattgtggagctaagtttggaccatggttagatgtacttgaaaatggtcctagttccaaatattatagttggtttatggtaaataagtggccttttgatgataataatcacgatacaaaggatggacgattttattcttttgcctttaatcagaaaatgccaaaattaaatacaaataatccagaagtaattgattatttaattaaggtatgtgagtattgggtaaaaaattataagattgatggattaagattagatgttgcaaatgaaatttcgcataagttctgtaagaagcttagagaaaaaatgaaatcgttaaatccagacttctatattttaggtgaaatatggcatgattctattccttggcttagaggtgatgaatttgatgctattatgaattattcactaactagtagtatatcagacttctggatagataagagtttaactaaggatgattttgagtacacaataaatagatgctatacaatatatatgcagcaaaataatgatgtgttatttaatttgttggattctcatgatacagaacgcttaatttcaagagtaaaagacattaacgtattttatcaacagctagctgtactatttacgatgccaggaagtccatgcatattttatggtacagaagttgcacttgaaggaaagtatgatcccgattgccgaagatgtatgccatgggatgaaataaaaagtggaatttatgatgataagattaatataatgaaggcgttgattaatttaagaaaagagcaaaaattatttagaagccgtaattttcattttccaaatacaattaaaaatagcagggtaatagaatatattaaaatagatgaaaatgggaataggttagaaattttactaaattgttcaaatatagatgttttaatagagaataatggtagtgttttgtttagtaatttatattctaataatagactgcttaaaaaaggtgtattaattaggaaggttgattctatataaggttcaatcaaataaataacaagtccgtttacatcatgggctgataaaaaatatccattttgcgatttgattttatttataaatgaaaaagatatttaattaaatcagcaatatgtacttattaattataaatgaaaaaataattttgaagaggagtagtcatggaattaacatataggttcggaagaggatactggagaaatataaaggaaggaaacgagagagaatggatgataggcaatggtattggcgggtatagcagtcaaactatcattaatagtggatttagatgtcataatgggtatttaatagcagcaatgaatccgccagtagaacgttattcaatattatatagaactcaggaaaaaatcgtcacagatggaagaacatatgatttgacttgtcaggaatataaggattatacgaagaatggttatgagtatctcaaaagttttatatttgattcagtgcctcaatatatttatcaaatagaagatataaatgtaaaaaaaactatagctatggaatatggatataatactgtagctatatgttatgagattgaaaatggaagttctaaggctaaaattgatattacaccactgtttaattttaaggaagctggtacatttaaggcttctgagcagctggattttaaaactgaattacaagacgatatattaaaattgtatcctaatgaagatgataagaagataataagttttatgtcatcagcaggcatatttaaggacagaagtcttataaaagtacagaatgattttaattataatccattaattgaagagaatcattactatgaatttgaaaatagaaatggatttattgggttaaataatcattatacgccatatgatattgaaattgaattagagccttttgaaactaaaaagttttatttaaaatgtacagtagaagagttaggtgataaagacggatttgatattgttaaagaatataaggaaagaacaaatgaattattgaatagatcaggctataaagatttttttgcattaaatttagtaaaagcagctgaccattttattgtagatagaaaaagtactggattgaaaacaatacttgcaggatttccttggtttgttgattgggggagagacactatgatagcttttgaaggtttaacgctgtgtacaaagagatttgaggatgcaagagaaatattaaagtcttttgcagaatatataaaagatggacttgttccaaatgtttttgcggataaaggaacacaagcgttttacaatactgcagatgcatcattatggtatatacaagctgtatataagtatttaaaatatactggaaagaaaagtgattttaagtttgttaatgataaattattcgacaagttaattgaaattattgatgcttattcaaatggcacacatttttcaataggtatggatgatgattgtcttattcatgctggcagcggattggatcaagtaacgtggatggatgtaagagtagacgaaatggttgttactccaaggcatggtaaaccagtagaaataaatgctctttggtataatgccctttgcataatggattggttatgtagaaagtatgaaatgaatggatcaaaatatgaaagtttagcgagaaaagttaaaaactcctttaacaaaaaattctggaatgaaaaagaacagtgtttatttgatgttgttgatgattatgatgggaaagttaggccaaatcaaatatgggcagtatcattgccatttactatgttagaaaaagaaaaggaagcgaaagttgtgaataaagtatataaagaattatattcgacttatggattgagatcgctgtcatacttagataaagattttaagagcgaatatataggaccacttatgaaaagggatttagcatatcatatggggacaacatgggcattcttaatagggagctttatatcagcatattgtaaggtaaataatcactctaaagaagcagtaagtagagcaaaagaaatgtgtgaagtatttcaggatcatatgaaagatggatgcataaatggaatagctgaagtatttgatggaaaattttcagctacaggcaggggatgctatagtcaagcctggagtgtaggcgaagttttaagagcatatactaacgatgtactgccatttatttgatctactttgca